European Patent Application EP 4 328 304 A2, published February 28, 2024. Title: ENGINEERED CLEAVAGE HALF-DOMAINS. Applicant: Sangamo Therapeutics, Inc. The sequence listing filed with the application follows.

SEQUENCE LISTING (57 sequences)

SEQ ID NO: 1 - protein, 7 aa, synthetic construct
  REGION 1..7: note = Description of Artificial Sequence: Synthetic peptide
RSDHLST

SEQ ID NO: 2 - protein, 7 aa, synthetic construct
  REGION 1..7: note = Description of Artificial Sequence: Synthetic peptide
TSANLSR

SEQ ID NO: 3 - protein, 7 aa, synthetic construct
  REGION 1..7: note = Description of Artificial Sequence: Synthetic peptide
RSDNLSE

SEQ ID NO: 4 - protein, 7 aa, synthetic construct
  REGION 1..7: note = Description of Artificial Sequence: Synthetic peptide
TSGSLTR

SEQ ID NO: 5 - protein, 7 aa, synthetic construct
  REGION 1..7: note = Description of Artificial Sequence: Synthetic peptide
QSGALAR

SEQ ID NO: 6 - protein, 7 aa, synthetic construct
  REGION 1..7: note = Description of Artificial Sequence: Synthetic peptide
RSDNLTR

SEQ ID NO: 7 - protein, 7 aa, synthetic construct
  REGION 1..7: note = Description of Artificial Sequence: Synthetic peptide
QSGNLAR

SEQ ID NO: 8 - protein, 7 aa, synthetic construct
  REGION 1..7: note = Description of Artificial Sequence: Synthetic peptide
QSGHLQR

SEQ ID NO: 9 - protein, 7 aa, synthetic construct
  REGION 1..7: note = Description of Artificial Sequence: Synthetic peptide
QSSDLRR

SEQ ID NO: 10 - protein, 7 aa, synthetic construct
  REGION 1..7: note = Description of Artificial Sequence: Synthetic peptide
RSDTLSE

SEQ ID NO: 11 - protein, 7 aa, synthetic construct
  REGION 1..7: note = Description of Artificial Sequence: Synthetic peptide
RSDNLSR

SEQ ID NO: 12 - protein, 7 aa, synthetic construct
  REGION 1..7: note = Description of Artificial Sequence: Synthetic peptide
QNAHRTT

SEQ ID NO: 13 - protein, 7 aa, synthetic construct
  REGION 1..7: note = Description of Artificial Sequence: Synthetic peptide
QSSNLAR

SEQ ID NO: 14 - protein, 7 aa, synthetic construct
  REGION 1..7: note = Description of Artificial Sequence: Synthetic peptide
RSDDLTR

SEQ ID NO: 15 - protein, 7 aa, synthetic construct
  REGION 1..7: note = Description of Artificial Sequence: Synthetic peptide
DRSHLSR

SEQ ID NO: 16 - protein, 7 aa, synthetic construct
  REGION 1..7: note = Description of Artificial Sequence: Synthetic peptide
DNPNLNR

SEQ ID NO: 17 - protein, 7 aa, synthetic construct
  REGION 1..7: note = Description of Artificial Sequence: Synthetic peptide
RSDDLSR

SEQ ID NO: 18 - protein, 7 aa, synthetic construct
  REGION 1..7: note = Description of Artificial Sequence: Synthetic peptide
RNAHRIN

SEQ ID NO: 19 - protein, 7 aa, synthetic construct
  REGION 1..7: note = Description of Artificial Sequence: Synthetic peptide
RSANLTR

SEQ ID NO: 20 - protein, 7 aa, synthetic construct
  REGION 1..7: note = Description of Artificial Sequence: Synthetic peptide
ASKTRKN

SEQ ID NO: 21 - protein, 7 aa, synthetic construct
  REGION 1..7: note = Description of Artificial Sequence: Synthetic peptide
DRSNLSR

SEQ ID NO: 22 - protein, 7 aa, synthetic construct
  REGION 1..7: note = Description of Artificial Sequence: Synthetic peptide
RSDHLSA

SEQ ID NO: 23 - protein, 7 aa, synthetic construct
  REGION 1..7: note = Description of Artificial Sequence: Synthetic peptide
QSGHLSR

SEQ ID NO: 24 - protein, 7 aa, synthetic construct
  REGION 1..7: note = Description of Artificial Sequence: Synthetic peptide
TSGSLSR

SEQ ID NO: 25 - protein, 7 aa, synthetic construct
  REGION 1..7: note = Description of Artificial Sequence: Synthetic peptide
RSDTLSA

SEQ ID NO: 26 - protein, 7 aa, synthetic construct
  REGION 1..7: note = Description of Artificial Sequence: Synthetic peptide
DNSNRIK

SEQ ID NO: 27 - protein, 7 aa, synthetic construct
  REGION 1..7: note = Description of Artificial Sequence: Synthetic peptide
RSAALSR

SEQ ID NO: 28 - protein, 7 aa, synthetic construct
  REGION 1..7: note = Description of Artificial Sequence: Synthetic peptide
QSGDLTR

SEQ ID NO: 29 - protein, 7 aa, synthetic construct
  REGION 1..7: note = Description of Artificial Sequence: Synthetic peptide
RSDSLSA

SEQ ID NO: 30 - protein, 7 aa, synthetic construct
  REGION 1..7: note = Description of Artificial Sequence: Synthetic peptide
DRSNLTR

SEQ ID NO: 31 - protein, 7 aa, synthetic construct
  REGION 1..7: note = Description of Artificial Sequence: Synthetic peptide
RSDNLSQ

SEQ ID NO: 32 - protein, 7 aa, synthetic construct
  REGION 1..7: note = Description of Artificial Sequence: Synthetic peptide
ASNDRKK

SEQ ID NO: 33 - protein, 7 aa, synthetic construct
  REGION 1..7: note = Description of Artificial Sequence: Synthetic peptide
DSSTRKK

SEQ ID NO: 34 - protein, 7 aa, synthetic construct
  REGION 1..7: note = Description of Artificial Sequence: Synthetic peptide
RSDNLSV

SEQ ID NO: 35 - protein, 7 aa, synthetic construct
  REGION 1..7: note = Description of Artificial Sequence: Synthetic peptide
DRSHLAR

SEQ ID NO: 36 - protein, 7 aa, synthetic construct
  REGION 1..7: note = Description of Artificial Sequence: Synthetic peptide
QRSNLVR

SEQ ID NO: 37 - protein, 7 aa, synthetic construct
  REGION 1..7: note = Description of Artificial Sequence: Synthetic peptide
QSSDLTR

SEQ ID NO: 38 - protein, 7 aa, synthetic construct
  REGION 1..7: note = Description of Artificial Sequence: Synthetic peptide
GNVDLIE

SEQ ID NO: 39 - protein, 7 aa, synthetic construct
  REGION 1..7: note = Description of Artificial Sequence: Synthetic peptide
RSSNLSR

SEQ ID NO: 40 - protein, 7 aa, synthetic construct
  REGION 1..7: note = Description of Artificial Sequence: Synthetic peptide
RSDSLSV

SEQ ID NO: 41 - protein, 7 aa, synthetic construct
  REGION 1..7: note = Description of Artificial Sequence: Synthetic peptide
TNHNRKT

SEQ ID NO: 42 - DNA, 28 bp, synthetic construct
  misc_feature 1..28: note = Description of Artificial Sequence: Synthetic oligonucleotide
  source 1..28: mol_type = other DNA
ttgttcaggattggacacaacatcctag

SEQ ID NO: 43 - DNA, 28 bp, synthetic construct
  misc_feature 1..28: note = Description of Artificial Sequence: Synthetic oligonucleotide
  source 1..28: mol_type = other DNA
cagctggagaagaacgaggagacggtaa

SEQ ID NO: 44 - DNA, 28 bp, synthetic construct
  misc_feature 1..28: note = Description of Artificial Sequence: Synthetic oligonucleotide
  source 1..28: mol_type = other DNA
ctgcggatagtgaggttccggttcccat

SEQ ID NO: 45 - DNA, 28 bp, synthetic construct
  misc_feature 1..28: note = Description of Artificial Sequence: Synthetic oligonucleotide
  source 1..28: mol_type = other DNA
tgaggaaggaggacgaaggcctctacac

SEQ ID NO: 46 - DNA, 28 bp, synthetic construct
  misc_feature 1..28: note = Description of Artificial Sequence: Synthetic oligonucleotide
  source 1..28: mol_type = other DNA
atgatgacgcccaggagcttcaccaccc

SEQ ID NO: 47 - DNA, 28 bp, synthetic construct
  misc_feature 1..28: note = Description of Artificial Sequence: Synthetic oligonucleotide
  source 1..28: mol_type = other DNA
gaggaagggaagtactccctggtgatgg

SEQ ID NO: 48 - DNA, 28 bp, synthetic construct
  misc_feature 1..28: note = Description of Artificial Sequence: Synthetic oligonucleotide
  source 1..28: mol_type = other DNA
gtgcagtgaaccaggctgttctgtggct

SEQ ID NO: 49 - DNA, 28 bp, synthetic construct
  misc_feature 1..28: note = Description of Artificial Sequence: Synthetic oligonucleotide
  source 1..28: mol_type = other DNA
gttcccagggacttgggatgggtcctgt

SEQ ID NO: 50 - DNA, 28 bp, synthetic construct
  misc_feature 1..28: note = Description of Artificial Sequence: Synthetic oligonucleotide
  source 1..28: mol_type = other DNA
aaggaggcaaggccgaggtctgcgatct

SEQ ID NO: 51 - DNA, 28 bp, synthetic construct
  misc_feature 1..28: note = Description of Artificial Sequence: Synthetic oligonucleotide
  source 1..28: mol_type = other DNA
aagatgtggagcaaactgaataatgaag

SEQ ID NO: 52 - DNA, 843 bp, synthetic construct
  misc_feature 1..843: note = Description of Artificial Sequence: Synthetic polynucleotide
  source 1..843: mol_type = other DNA
ggaagttaaagcccatgtttctaatacaatgaacattatgttatgcccaaacttaacaccatcatttcatatgatagcactttcttatagtgttaccttatgctccctgaccaaactcccagacatcaacttgtacttttctattttattctagatctttttgtattgttgttttaaatactttcctgcccattagaggacctaggagccaccctcctctcccctcttaactgatatttagcctttcatgggctttgcatataatggaaatttcaaaatccaccctgagaaatgaaaaccaagtagaggaaaaataaactcttcaaaacacacactaccttccactgctcttttgaagaaaactttacagcttccacaagttaagactccataatgacatcctgaagcttcatcagagcacaccaggcagagtttgggaggtggtcctgttgttgaggcatccagtccagacgggatccagccatactcactgctgttgaggagctggatggaggagagcttacatctggtctcatgctggggctaaagaaggggaagaacagtgttatgatttaactgtcaaaggaatatcaaaatacagttctcttagcttctcacttcatagtcagaatgctcacagtgaactctggcttcaagtgctagcaggcactaaaatatcctagctaaatatattcaaatcatgttatattcttctttaaacaaaattaagaatgaggtcatttcttttgaagtgtctccaaaatagaatggtgtggttctggttcacttcttcttctttttttttttttttttagatgcttaggatttatttttataatcacg

SEQ ID NO: 53 - DNA, 32 bp, synthetic construct
  misc_feature 1..32: note = Description of Artificial Sequence: Synthetic oligonucleotide
  source 1..32: mol_type = other DNA
catcatcctcatcttcagccacctgtgggcgg

SEQ ID NO: 54 - DNA, 32 bp, synthetic construct
  misc_feature 1..32: note = Description of Artificial Sequence: Synthetic oligonucleotide
  source 1..32: mol_type = other DNA
ggcaatactcatcttcactgacctgagggtgg

SEQ ID NO: 55 - DNA, 31 bp, synthetic construct
  misc_feature 1..31: note = Description of Artificial Sequence: Synthetic oligonucleotide
  source 1..31: mol_type = other DNA
actcccctacttcaacataaactgcaaaagg

SEQ ID NO: 56 - DNA, 31 bp, synthetic construct
  misc_feature 1..31: note = Description of Artificial Sequence: Synthetic oligonucleotide
  source 1..31: mol_type = other DNA
agacaccttcaactgcttaaactgaaaaagg

SEQ ID NO: 57 - protein, 579 aa, Flavobacterium okeanokoites
  REGION 1..579: note = FokI sequence
MVSKIRTFGWVQNPGKFENLKRVVQVFDRNSKVHNEVKNIKIPTLVKESKIQKELVAIMNQHDLIYTYKELVGTGTSIRSEAPCDAIIQATIADQGNKKGYIDNWSSDGFLRWAHALGFIEYINKSDSFVITDVGLAYSKSADGSAIEKEILIEAISSYPPAIRILTLLEDGQHLTKFDLGKNLGFSGESGFTSLPEGILLDTLANAMPKDKGEIRNNWEGSSDKYARMIGGWLDKLGLVKQGKKEFIIPTLGKPDNKEFISHAFKITGEGLKVLRRAKGSTKFTRVPKRVYWEMLATNLTDKEYVRTRRALILEILIKAGSLKIEQIQDNLKKLGFDEVIETIENDIKGLINTGIFIEIKGRFYQLKDHILQFVIPNRLGKPQLVKSELEEKKSELRHKLKYVPHEYIELIEIARNSTQDRILEMKVMEFFMKVYGYRGKHLGGSRKPDGAIYTVGSPIDYGVIVDTKAYSGGYNLPIGQADEMQRYVEENQTRNKHINPNEWWKVYPSSVTEFKFLFVSGHFKGNYKAQLTRLNHITNCNGAVLSVEELLIGGEMIKAGTLTLEEVRRKFNNGEINF